European Patent Application EP 4 378 472 A1, published June 5, 2024. Title: A therapeutic agent for an ischemic disease. Applicant: 宮崎　徹. The sequence listing filed with the application follows.

SEQUENCE LISTING (24 sequences)

SEQ ID NO: 1 - protein, 347 aa, Homo sapiens
MALLFSLILAICTRPGFLASPSGVRLVGGLHRCEGRVEVEQKGQWGTVCDDGWDIKDVAVLCRELGCGAASGTPSGILYEPPAEKEQKVLIQSVSCTGTEDTLAQCEQEEVYDCSHDEDAGASCENPESSFSPVPEGVRLADGPGHCKGRVEVKHQNQWYTVCQTGWSLRAAKVVCRQLGCGRAVLTQKRCNKHAYGRKPIWLSQMSCSGREATLQDCPSGPWGKNTCNHDEDTWVECEDPFDLRLVGGDNLCSGRLEVLHKGVWGSVCDDNWGEKEDQVVCKQLGCGKSLSPSFRDRKCYGPGVGRIWLDNVRCSGEEQSLEQCQHRFWGFHDCTHQEDVAVICSG

SEQ ID NO: 2 - DNA, 1044 bp, Homo sapiens
  source 1..1044: mol_type = other DNA; note = cDNA of human AIM
atggctctgctattctccttgatccttgccatttgcaccagacctggattcctagcgtctccatctggagtgcggctggtggggggcctccaccgctgtgaagggcgggtggaggtggaacagaaaggccagtggggcaccgtgtgtgatgacggctgggacattaaggacgtggctgtgttgtgccgggagctgggctgtggagctgccagcggaacccctagtggtattttgtatgagccaccagcagaaaaagagcaaaaggtcctcatccaatcagtcagttgcacaggaacagaagatacattggctcagtgtgagcaagaagaagtttatgattgttcacatgatgaagatgctggggcatcgtgtgagaacccagagagctctttctccccagtcccagagggtgtcaggctggctgacggccctgggcattgcaagggacgcgtggaagtgaagcaccagaaccagtggtataccgtgtgccagacaggctggagcctccgggccgcaaaggtggtgtgccggcagctgggatgtgggagggctgtactgactcaaaaacgctgcaacaagcatgcctatggccgaaaacccatctggctgagccagatgtcatgctcaggacgagaagcaacccttcaggattgcccttctgggccttgggggaagaacacctgcaaccatgatgaagacacgtgggtcgaatgtgaagatccctttgacttgagactagtaggaggagacaacctctgctctgggcgactggaggtgctgcacaagggcgtatggggctctgtctgtgatgacaactggggagaaaaggaggaccaggtggtatgcaagcaactgggctgtgggaagtccctctctccctccttcagagaccggaaatgctatggccctggggttggccgcatctggctggataatgttcgttgctcaggggaggagcagtccctggagcagtgccagcacagattttgggggtttcacgactgcacccaccaggaagatgtggctgtcatctgctcaggatag

SEQ ID NO: 3 - DNA, 24 bp, synthetic construct
  misc_feature 1..24: note = partial sequence in pX335 vector
  source 1..24: mol_type = other DNA
caccgaacaatggagccatggccc

SEQ ID NO: 4 - DNA, 24 bp, synthetic construct
  misc_feature 1..24: note = partial sequence in pX335 vector
  source 1..24: mol_type = other DNA
caccggtgagtgtccctgcttctg

SEQ ID NO: 5 - DNA, 20 bp, synthetic construct
  misc_feature 1..20: note = quantitative PCR primer for f-GAPDH
  source 1..20: mol_type = other DNA
agaacatcatccctgcattc

SEQ ID NO: 6 - DNA, 20 bp, synthetic construct
  misc_feature 1..20: note = quantitative PCR primer for r-GAPDH
  source 1..20: mol_type = other DNA
cacattgggggtaggaacac

SEQ ID NO: 7 - DNA, 21 bp, synthetic construct
  misc_feature 1..21: note = quantitative PCR primer for f-mAIM
  source 1..21: mol_type = other DNA
gaggacacatggatggaatgt

SEQ ID NO: 8 - DNA, 20 bp, synthetic construct
  misc_feature 1..20: note = quantitative PCR primer for r-mAIM
  source 1..20: mol_type = other DNA
acccttgtgtagcacctcca

SEQ ID NO: 9 - DNA, 20 bp, synthetic construct
  misc_feature 1..20: note = quantitative PCR primer for f-IL1B
  source 1..20: mol_type = other DNA
caggcaggcagtatcactca

SEQ ID NO: 10 - DNA, 20 bp, synthetic construct
  misc_feature 1..20: note = quantitative PCR primer for r-IL1B
  source 1..20: mol_type = other DNA
aggccacaggtattttgtcg

SEQ ID NO: 11 - DNA, 21 bp, synthetic construct
  misc_feature 1..21: note = quantitative PCR primer for f-IL6
  source 1..21: mol_type = other DNA
atggatgctaccaaactggat

SEQ ID NO: 12 - DNA, 21 bp, synthetic construct
  misc_feature 1..21: note = quantitative PCR primer for r-IL6
  source 1..21: mol_type = other DNA
tgaaggactctggctttgtct

SEQ ID NO: 13 - DNA, 22 bp, synthetic construct
  misc_feature 1..22: note = quantitative PCR primer for f-TNFA
  source 1..22: mol_type = other DNA
cttctgtctactgaacttcggg

SEQ ID NO: 14 - DNA, 21 bp, synthetic construct
  misc_feature 1..21: note = quantitative PCR primer for r-TNFA
  source 1..21: mol_type = other DNA
tgatctgagtgtgagggtctg

SEQ ID NO: 15 - DNA, 19 bp, synthetic construct
  misc_feature 1..19: note = quantitative PCR primer for f-IL23
  source 1..19: mol_type = other DNA
caacttcacacctccctac

SEQ ID NO: 16 - DNA, 18 bp, synthetic construct
  misc_feature 1..18: note = quantitative PCR primer for r-IL23
  source 1..18: mol_type = other DNA
ccactgctgactagaact

SEQ ID NO: 17 - DNA, 18 bp, synthetic construct
  misc_feature 1..18: note = quantitative PCR primer for f-MCP1
  source 1..18: mol_type = other DNA
catccacgtgttggctca

SEQ ID NO: 18 - DNA, 23 bp, synthetic construct
  misc_feature 1..23: note = quantitative PCR primer for r-MCP1
  source 1..23: mol_type = other DNA
gatcatcttgctggtgaatgagt

SEQ ID NO: 19 - DNA, 20 bp, synthetic construct
  misc_feature 1..20: note = quantitative PCR primer for f-CD11b
  source 1..20: mol_type = other DNA
caatagccagcctcagtgcc

SEQ ID NO: 20 - DNA, 19 bp, synthetic construct
  misc_feature 1..19: note = quantitative PCR primer for r-CD11b
  source 1..19: mol_type = other DNA
gagcccaggggagaagtgg

SEQ ID NO: 21 - DNA, 20 bp, synthetic construct
  misc_feature 1..20: note = quantitative PCR primer for f-beta-actin
  source 1..20: mol_type = other DNA
ctaaggccaaccgtgaaaag

SEQ ID NO: 22 - DNA, 20 bp, synthetic construct
  misc_feature 1..20: note = quantitative PCR primer for r-beta-actin
  source 1..20: mol_type = other DNA
accagaggcatacagggaca

SEQ ID NO: 23 - DNA, 21 bp, synthetic construct
  misc_feature 1..21: note = quantitative PCR primer for f-18SrRNA
  source 1..21: mol_type = other DNA
cgccgctagaggtgaaattct

SEQ ID NO: 24 - DNA, 21 bp, synthetic construct
  misc_feature 1..21: note = quantitative PCR primer for r-18SrRNA
  source 1..21: mol_type = other DNA
cattcttggcaaatgctttcg